European Patent Specification EP 3 475 417 B1, published May 24, 2023. Title: COMPOSITIONS AND METHODS FOR MAKING BENZYLISOQUINOLINE ALKALOIDS, MORPHINAN ALKALOIDS, THEBAINE, AND DERIVATIVES THEREOF. Applicant: Facchini, Peter J Chen, Xue. The sequence listing filed with the application follows.

SEQUENCE LISTING (81 sequences)

SEQ ID NO: 1 - DNA, 1425 bp, Papaver somniferum
atggcaacaatgtatagtgctgctgttgaagtgatctctaaggaaaccattaaacccacaactccaaccccatctcaacttaaaaacttcaatctgtcacttctcgatcaatgttttcctttatattattatgttccaatcattcttttctacccagccaccgccgctaatagtaccggtagcagtaaccatcatgatgatcttgacttgcttaagagttctctttccaaaacactagttcacttttatccaatggctggtaggatgatagacaatattctggtcgactgtcatgaccaagggattaacttttacaaagttaaaattagaggtaaaatgtgtgagttcatgtcgcaaccggatgtgccactaagccagcttcttccctctgaagttgtttccgcgagtgtccctaaggaagcactggtgatcgttcaagtgaacatgtttgactgtggtggaacagccatttgttcgagtgtatcacataagattgccgatgcagctacaatgagtacgttcattcgtagttgggcaagcaccactaaaacatctcgtagtgggggttcaactgctgccgttacagatcagaaattgattccttctttcgactcggcatctctattcccacctagtgaacgattgacatctccatcagggatgtcagagataccattttccagtaccccagaggatacagaagatgataaaactgtcagcaagagatttgtgttcgattttgcaaagataacatctgtacgtgaaaagttgcaagtattgatgcatgataactacaaaagccgcaggcaaacaagggttgaggtggttacttctctaatatggaagtccgtgatgaaatccactccagccggttttttaccagtggtacatcatgccgtgaaccttagaaagaaaatggacccaccattacaagatgtttcattcggaaatctatctgtaactgtttcggcgttcttaccagcaacaacaacgacaacaacaaatgcggtcaacaagacaatcaatagtacgagtagtgaatcacaagtggtacttcatgagttacatgattttatagctcagatgaggagtgaaatagataaggtcaagggtgataaaggtagcttggagaaagtcattcaaaattttgcttctggtcatgatgcttcaataaagaaaatcaatgatgttgaagtgataaacttttggataagtagctggtgcaggatgggattatacgagattgattttggttggggaaagccaatttgggtaacagttgatccaaatatcaagccgaacaagaattgttttttcatgaatgatacgaaatgtggtgaaggaatagaagtttgggcgagctttcttgaggatgatatggctaagttcgagcttcacctaagtgaaatccttgaattgatttga

SEQ ID NO: 2 - protein, 474 aa, Papaver somniferum
MATMYSAAVEVISKETIKPTTPTPSQLKNFNLSLLDQCFPLYYYVPIILFYPATAANSTGSSNHHDDLDLLKSSLSKTLVHFYPMAGRMIDNILVDCHDQGINFYKVKIRGKMCEFMSQPDVPLSQLLPSEVVSASVPKEALVIVQVNMFDCGGTAICSSVSHKIADAATMSTFIRSWASTTKTSRSGGSTAAVTDQKLIPSFDSASLFPPSERLTSPSGMSEIPFSSTPEDTEDDKTVSKRFVFDFAKITSVREKLQVLMHDNYKSRRQTRVEVVTSLIWKSVMKSTPAGFLPVVHHAVNLRKKMDPPLQDVSFGNLSVTVSAFLPATTTTTTNAVNKTINSTSSESQVVLHELHDFIAQMRSEIDKVKGDKGSLEKVIQNFASGHDASIKKINDVEVINFWISSWCRMGLYEIDFGWGKPIWVTVDPNIKPNKNCFFMNDTKCGEGIEVWASFLEDDMAKFELHLSEILELI

SEQ ID NO: 3 - DNA, 936 bp, Papaver somniferum
atgcctgaaacatgtccaaatactgttacaaagaggaggtgtgcagttgttactggcggaaacaagggtatcggatttgagatttgtaagcaattatcttctaatggaatcatggttgttttaacttgtagagatgtaactaaaggtcatgaagctgttgaaaaactcaaaaattccaatcatgagaatgtggtttttcatcaacttgatgttacggatccaattgctactatgtcttctttagcggatttcattaaaacacacttcggaaagcttgatatcttggtaaacaatgctggggttgcaggtttttcagttgatgctgatcgttttaaggcaatgataagtgacattggagaggattcagaggagctcgtgaagatctacgaaaaaccagaagcccaagaattaatgtcagagacatatgaattagcagaagaatgtctcaaaataaattacaacggtgttaaatcggtaaccgaagttctaattcctttacttcaactatctgattcaccaagaattgttaatgtttcatcatccacgggaagcctcaagtatgtatccaatgaaacagctctagagatacttggagatggtgatgcattaacagaagagagaattgacatggtagtgaatatgcttcttaaggattttaaggaaaatttgatcgaaacaaatgggtggcctagtttcggagctgcatacacaacatcaaaagcatgtttgaatgcttacacaagggtgttagcaaacaaaattcccaaatttcaggtcaattgtgtttgtcctggtttggttaaaacagaaatgaactacggcattggaaattatactgccgaagaaggtgctgaacatgtagtcagaatagctcttttccccgacgatggaccttctggttttttctatgattgttcagaactatctgcattttga

SEQ ID NO: 4 - protein, 311 aa, Papaver somniferum
MPETCPNTVTKRRCAVVTGGNKGIGFEICKQLSSNGIMVVLTCRDVTKGHEAVEKLKNSNHENVVFHQLDVTDPIATMSSLADFIKTHFGKLDILVNNAGVAGFSVDADRFKAMISDIGEDSEELVKIYEKPEAQELMSETYELAEECLKINYNGVKSVTEVLIPLLQLSDSPRIVNVSSSTGSLKYVSNETALEILGDGDALTEERIDMVVNMLLKDFKENLIETNGWPSFGAAYTTSKACLNAYTRVLANKIPKFQVNCVCPGLVKTEMNYGIGNYTAEEGAEHVVRIALFPDDGPSGFFYDCSELSAF

SEQ ID NO: 5 - protein, 158 aa, Papaver somniferum
MAHHGVSGLVGKIVTELEVNCNADEFYKILKRDEDVPRAVSDLFPPVKIAKGDGLVSGCIKEWDCVLDGKAMSGKEETTHNDETRTLRHRELEGDLMKDYKKFDSIIEVNPKPNGHGSIVTWSIEYEKMNEDSPAPFAYLASFHQNVVEVDSHLCLSE

SEQ ID NO: 6 - protein, 160 aa, Papaver somniferum
MAPLGVSGLVGKLSTELEVDCDAEKYYNMYKHGEDVKKAVPHLCVDVKIISGDPTSSGCIKEWNVNIDGKTIRSVEETTHDDETKTLRHRVFEGDVMKDFKKFDTIMVVNPKPDGNGCVVTRSIEYEKTNENSPTPFDYLQFGHQAIEDMNKYLRDSESN

SEQ ID NO: 7 - protein, 157 aa, Papaver somniferum
MAHHGVSGLVGKLVTELEVHCNADAYYKIFKHQEDVPKAMPHLYTGGKVISGDATRSGCIKEWNYILEGKALIAVEETTHDDETRTLTHRITGGDLTKDYKKFVKIVEVNPKPNGHGSIVTVSLVYEKMNEGSPTPFNYLQFVHQTIVGLNSHICAS

SEQ ID NO: 8 - protein, 159 aa, Papaver somniferum
MAHPHPISGLVGKLVTELEVNCDADKYYKIFKHHEDVPKAVPHMYTSVKVVEGHGITSGCVKEWGYLLEGKELIVKETTTYTDETRTIHHSAVGGHMTKIYKKFDATLVVNPKPSGHGSTVSWTIDYEKINEDSPVPIPYLAFFHKLIEDLNSHLCASD

SEQ ID NO: 9 - protein, 159 aa, Papaver somniferum
MAHQHTISGLVGKLITESEVNCNADKYYQIFKHHEDLPSAIPHIYTSVKAVEGHGTTSGCVKEWCYILEGKPLTVKEKTTYNDETRTINHNGIEGGMMTDYKKFVATLVVKPKANGQGSIVTWIVDYEKINEDSPVPFDYLAFFQQNIEDLNSHLCASD

SEQ ID NO: 10 - protein, 164 aa, Papaver somniferum
MRYEFINEFDAHASADDVWGGIYGSIDYPKLVVQLLPTVLEKKEILEGDGHNVGTVLHVVYLPGFVPRTYNEKIVTMDHKKRYKEVQMVEGGYLDMGFTYVMVIHEVLAKECNSCIIRSIVKCEVKDEFAANVSNIRNTFDGYVALARAVPEYIAKQHATSAAN

SEQ ID NO: 11 - protein, 159 aa, Papaver somniferum
MAHAHGISGLVGKLITESEVNCNADKFYQMFKHDENITNIIPHIYTSFKVVEGDGLISGCTKEWGYLSEGKARIVKEQTTFDDETRTIHHCAKAGDMMNDYKKFVLTLVVNPKAHGQGSTVKWIIDYEKINEDSPVPFAYLSLCIKITEGLNSHIYASE

SEQ ID NO: 12 - protein, 157 aa, Papaver somniferum
MAQHHTISGLIGKLVTESEVNCDAEKYYKIIKHHEDVPNATPYVSDVKVTEGHGTTSGCVKQWNFVVAGRNEYVLEKTTYNDETRTICHSDFEGDLMKKYKKFDAILVVKPKDNGHGSNVRWTIEYEKNNEDSPVPIDYLGFFQSLIDDLNSHLCSS

SEQ ID NO: 13 - protein, 180 aa, Papaver somniferum
MDSINSSIYFCAYFRELIIKLLMAPLGVSGLVGKLSTELEVDCDAEKYYNMYKHGEDVQKAVPHLCVDVKVISGDPTSSGCIKEWNVNIDGKTIRSVEETTHNDETKTLRHRVFEGDMMKDFKKFDTIMVVNPKPDGNGCVVTRSIEYEKTNENSPTPFDYLQFGHQAIEDMNKYLRDSE

SEQ ID NO: 14 - protein, 160 aa, Papaver somniferum; identical to SEQ ID NO: 6

SEQ ID NO: 15 - protein, 132 aa, Papaver somniferum
MYKHGEDVKKAVPHLCVDVKIISGDPTSSGCIKEWNVNIDGKTIRSVEETTHDDETKTLRHRVFEGDVMKDFKKFDTIMVVNPKPDGNGCVVTRSIEYEKTNENSPTPFDYLQFGHQAIEDMNKYLRDSESN

SEQ ID NO: 16 - protein, 127 aa, Papaver somniferum
MDSINSSIYFCAYFRELIIKLLMAPPGVSGLVGKLSTELDVNCDAEKYYNMYKHGEDVQKAVPHLCVDVKVISGDPTRSGCIKEWNVNIGNVQTHYCNSSIYFTCFWFSVHHYIYILTIAVIYFTLN

SEQ ID NO: 17 - protein, 108 aa, Papaver somniferum
MSIAMLKNIITCISTEKMCKRQFLIFALTSKLSVETQPVQVVSRNGMLTSVMYKHTIAIHQFTSHAFGSPCIIIYIYSQLQSYISRLIRFDLGFTTLRYNVCLHACRW

SEQ ID NO: 18 - DNA, 477 bp, Papaver somniferum
atggcgcatcatggtgtttcaggtctagttgggaaaattgtaactgaattggaggtgaattgtaatgccgacgaattttataagattttgaagcgcgatgaagatgttccacgggcagtttctgatcttttccctcccgtcaaaattgccaaaggagatggacttgtttctggttgtatcaaggaatgggactgtgttcttgatggtaaggcgatgagcggcaaggaggaaacaacacacaacgatgaaacgaggactttgcgtcaccgtgaattggaaggagacttgatgaaggattacaagaagtttgattccataattgaagttaatccaaaaccaaatggacatggaagcattgtgacgtggtcaattgagtatgagaaaatgaacgaagattctccggctccctttgcttatctagcttccttccatcagaacgttgtggaagttgattctcacctctgcctttctgaataa

SEQ ID NO: 19 - DNA, 483 bp, Papaver somniferum
atggctcctctcggtgtttcaggtttagtcgggaaactttcaactgaattggaggtcgattgcgatgctgaaaaatattataacatgtataagcacggagaagatgtaaaaaaggcagttcctcatctttgcgttgacgtcaaaattatcagtggagatccgaccagttcaggttgtatcaaggaatggaatgttaacattgatggtaagacgattcgctcggtagaggaaaccacacacgatgatgaaacgaaaacgttacgtcaccgtgtatttgaaggagacgtgatgaaggatttcaagaagtttgatacgataatggtagtcaatccaaagccggatggaaatggatgtgttgtgacaaggtcaattgagtatgaaaaaaccaacgagaattctccaactccctttgattatctacaattcggccatcaggccattgaggacatgaacaagtacttacgcgattctgaaagtaactga

SEQ ID NO: 20 - DNA, 474 bp, Papaver somniferum
atggcgcatcatggtgtttcaggtctagttgggaaacttgtaactgaattggaggtccattgcaatgctgacgcatactataaaatctttaagcaccaagaagatgtaccaaaggcaatgcctcatctttacactggcgggaaagttatcagtggagatgcaacccgttctggttgtatcaaggaatggaactacattcttgagggtaaggcgctgatcgcagtggaggaaacaacacatgacgatgaaacaaggaccttaacacaccgcataactggaggagacttgacaaaggattacaaaaagttcgttaagatcgttgaagttaatccaaagcctaatggacatggaagcattgtgactgtatcccttgtgtatgagaaaatgaacgagggttctccaactccctttaattatctacaatttgtccatcagaccattgtaggcttgaattctcacatctgcgcttcttag

SEQ ID NO: 21 - DNA, 480 bp, Papaver somniferum
atggctcatccccatcctatttcaggtctagttgggaaactagtgactgaattggaggttaactgcgacgctgacaagtattacaaaatttttaagcaccatgaagatgttccaaaagcagtacctcatatgtacactagcgtcaaagttgtcgagggacatggaattacttctggttgtgtcaaggaatggggttatcttcttgagggaaaagaactgattgtcaaggaaacaacaacatacactgatgaaacaaggacgatacatcatagcgcagtaggaggacacatgacgaagatttacaagaagtttgatgcaacgcttgtagtcaatccaaagcctagtggccatggaagcacggtgagttggactattgattatgagaaaattaacgaggattctcccgttcctattccatatctagctttcttccataagctcatcgaggacttgaactctcacctctgcgcttctgattaa

SEQ ID NO: 22 - DNA, 480 bp, Papaver somniferum
atggcccatcaacatacaatttcaggtcttgtgggaaaacttattactgaatcggaggttaactgcaatgccgacaagtattaccaaatatttaagcaccatgaagaccttccaagcgcaatccctcatatttacactagcgtcaaagctgtcgagggacatggaactacttctggatgtgtcaaggagtggtgctatattcttgaggggaaaccacttacagttaaggagaaaacaacgtacaatgatgaaacaagaacgataaatcataatggaatagaaggaggcatgatgactgattacaagaagttcgttgcaacacttgtagttaagccaaaagctaatgggcaaggaagcatcgtgacatggatagtggattatgagaagattaatgaggattctccagttcctttcgactatctagctttcttccaacaaaacatcgaagacttgaactctcacctctgtgcttctgattaa

SEQ ID NO: 23 - DNA, 495 bp, Papaver somniferum
atgaggtacgagtttataaacgagtttgatgcacatgcatcagcagacgatgtttggggaggaatctatggctccattgattaccctaaactagtggttcaattacttccaactgtcctcgaaaagaaggaaatcttggaaggcgatggtcataatgttggtactgttctgcatgttgtgtaccttccaggatttgttccgcggacgtacaacgagaagattgtaacgatggatcacaaaaaacgttacaaggaagtacaaatggttgaaggaggatacttggatatgggatttacatatgtcatggtaattcatgaagtactagcaaaagaatgtaattcttgtatcattagatcaattgttaagtgtgaagtcaaggatgaatttgctgcaaatgtttctaatattcgcaacacctttgatggatatgtcgccttagcccgagccgttccggaatatattgcgaagcagcacgcaacatcagcagctaattaa

SEQ ID NO: 24 - DNA, 480 bp, Papaver somniferum
atggctcatgctcatggtatttcaggtctagttgggaaacttattactgaatcggaggttaactgcaacgctgacaagttttaccaaatgtttaagcacgatgaaaatattacaaatataattcctcatatctatactagtttcaaggttgtcgagggagatggacttatttctggttgtaccaaggaatggggctatctttctgagggcaaagcaaggattgttaaggagcaaacgacctttgatgacgaaacaaggacgatacatcattgcgcaaaagcaggagacatgatgaatgattacaagaagttcgttctaacacttgtagttaatccaaaggctcatggacaaggaagcacagtcaagtggattatagattatgagaagataaatgaggattctccagttccttttgcttatctatctctgtgcattaagatcactgaaggtctgaactctcacatctacgcttccgaatag

SEQ ID NO: 25 - DNA, 474 bp, Papaver somniferum
atggctcaacatcataccatttcaggtcttattgggaagcttgtgaccgaatcagaagttaattgcgatgctgaaaaatattacaaaataattaagcaccacgaagatgtacctaatgcaaccccttatgtttccgatgtcaaagttactgaaggacatggtaccacttcgggttgtgtcaagcaatggaactttgttgttgcgggtcgaaacgaatatgtccttgaaaaaacaacatacaatgatgaaacaaggacaatatgtcacagtgactttgaaggagacctgatgaagaaatacaagaagtttgatgcaatccttgtagttaagccaaaggataatggacatggtagtaatgtgagatggactattgaatatgagaagaataacgaggattctccggttccaattgattatctaggtttcttccaatcgttaatcgatgacttgaactctcatctttgctcctcttaa

SEQ ID NO: 26 - DNA, 543 bp, Papaver somniferum
atggattctattaattcttccatatacttctgtgcatattttagagaactaatcatcaaattgttgatggctcctcttggtgtttcaggtttagtcgggaaactttcaactgaattggaggtcgattgcgatgctgaaaaatattataacatgtataagcacggagaagatgtgcaaaaggcagttcctcatctttgcgttgacgtcaaagttatcagtggagatccgaccagttcaggttgtatcaaggaatggaatgttaacattgatggtaagacgattcgctcagtagaggaaacaacacacaatgatgaaacgaaaacgttgcgtcaccgtgtatttgaaggagacatgatgaaggatttcaagaagtttgatacgataatggtagtcaatccaaagccggatggaaatggatgtgttgtgacacggtcaattgagtatgagaaaaccaacgagaattctccgactccctttgattatctacaattcggccatcaggccattgaagacatgaacaaatacttacgcgattctgaataa

SEQ ID NO: 27 - DNA, 483 bp, Papaver somniferum
atggctcctctcggtgtttcaggtttagtcgggaaactttcaactgaattggaggtcgattgcgatgctgaaaaatattataacatgtataagcacggagaagatgtaaaaaaggcagttcctcatctttgcgttgacgtcaaaattatcagtggagatccgaccagttcaggttgtatcaaggaatggaatgttaacattgatggtaagacgattcgctcggtagaggaaaccacacacgatgatgaaacgaaaacgttacgtcaccgtgtatttgaaggagacgtgatgaaggatttcaagaagtttgatacgataatggtagtcaatccaaagccggatggaaatggatgtgttgtgacaaggtcaattgagtatgagaaaaccaacgagaattctccaactccctttgattatctacaattcggccatcaggccattgaggacatgaacaagtacttacgcgattctgaaagtaactga

SEQ ID NO: 28 - DNA, 399 bp, Papaver somniferum
atgtataagcacggagaagatgtaaaaaaggcagttcctcatctttgcgttgacgtcaaaattatcagtggagatccgaccagttcaggttgtatcaaggaatggaatgttaacattgatggtaagacgattcgctcggtagaggaaaccacacacgatgatgaaacgaaaacgttacgtcaccgtgtatttgaaggagacgtgatgaaggatttcaagaagtttgatacgataatggtagtcaatccaaagccggatggaaatggatgtgttgtgacaaggtcaattgagtatgaaaaaaccaacgagaattctccaactccctttgattatctacaattcggccatcaggccattgaggacatgaacaagtacttacgcgattctgaaagtaactga

SEQ ID NO: 29 - DNA, 384 bp, Papaver somniferum
atggattctattaattcttccatatacttctgtgcatattttagagaactaatcattaaattgttgatggctcctcctggtgtttcaggtctagtcgggaaactttcaactgaattggatgtcaattgcgatgctgaaaaatattataacatgtataagcacggagaagatgtgcaaaaggcagttcctcatctttgcgttgacgtcaaagttatcagtggagacccaacccgttcaggttgtatcaaggaatggaatgttaacatcggtaatgtacaaacacactattgcaattcatcaatttacttcacatgcttttggttctccgtgcatcattatatatatatactcacaattgcagtcatatatttcacgcttaattag

SEQ ID NO: 30 - DNA, 327 bp, Papaver somniferum
atgtcaattgcgatgctgaaaaatattataacatgtataagcacggagaagatgtgcaaaaggcagttcctcatctttgcgttgacgtcaaagttatcagtggagacccaacccgttcaggttgtatcaaggaatggaatgttaacatcggtaatgtacaaacacactattgcaattcatcaatttacttcacatgcttttggttctccgtgcatcattatatatatatactcacaattgcagtcatatatttcacgcttaattagatttgatttgggtttcacaactttgcggtataatgtttgtcttcacgcatgcagatggtaa

SEQ ID NO: 31 - protein, 180 aa, Papaver somniferum
MDSINSSIYFCAYFRELIIKLLMAPLGVSGLVGKLSTELEVDCDAEKYYNMYKHGEDVKKAVPHLCVDVKIISGDPTSSGCIKEWNVNIDGKTIRSVEETTHDDETKTLRHRVFEGDVMKDFKKFDTIMVVNPKPDGNGCVVTRSIEYEKTNENSPTPFDYLQFGHQAIEDMNKYLRDSE

SEQ ID NO: 32 - protein, 132 aa, Papaver somniferum; identical to SEQ ID NO: 15

SEQ ID NO: 33 - protein, 166 aa, Papaver somniferum
MAHHGVSGLVGKIVTELEVNCNADEFYKILKRDEDVPRAVSDLFPPVKIAKGDGLVSGCIKEWDCVLDGKAMSGKEETTHNDETRTLRHRELEGDLMKDYKKFDSIIEVNPKPNGHGSIVTWSIEYEKMNEDSPAPFAYLASFHQNVVEVDSHLCLSEDYKDDDDK

SEQ ID NO: 34 - protein, 167 aa, Papaver somniferum
MDYKDDDDKMAHHGVSGLVGKIVTELEVNCNADEFYKILKRDEDVPRAVSDLFPPVKIAKGDGLVSGCIKEWDCVLDGKAMSGKEETTHNDETRTLRHRELEGDLMKDYKKFDSIIEVNPKPNGHGSIVTWSIEYEKMNEDSPAPFAYLASFHQNVVEVDSHLCLSE

SEQ ID NO: 35 - protein, 384 aa, Papaver somniferum
MIIETLDILGPNQNGNSGTHTQKPIKTRNWLLIIINCALVFCGVIGGPLLMRLYYLHGGSRKWLSSFLQTAGFPVLIFPLIFLYIKPKLSTQNNDQSSSFFMEPKLFLWSAIVGIVFGVSNFMYALGLSYLPVSTSTILFATQLCFTAIFAWLIVKQKFTAFIINAVIVMTLGSILLGINTNGDRPIGVSKTQYLIGFLMTLAAAALTGLGTPFVELSFIKATRNITYPTLLQFQVILCLFGTCLNVIGMLINKDFQAIPREADMFELGKSKYYMIICLTALTWQLSGIGLVGLILYTNALFNGIYVSVLVPFTEVAAVIFFHEKFTGLKGMALALCLWGFSSYFYGEYKMMNKVGDNETHEKIEEAESEPKRLEDQQAPYSTV

SEQ ID NO: 36 - DNA, 1155 bp, Papaver somniferum
atgatcatcgaaacactagatatcctgggaccaaatcagaatggcaattcaggaacccatactcaaaaaccaatcaaaaccagaaactggctgctgatcattattaactgcgccttagttttttgtggtgttataggtggtcctctcttaatgagactgtactatcttcatggtggtagtcgtaaatggcttagtagttttctgcaaactgctggtttcccagttctcatatttcctctcatttttctctacattaaaccgaaattgtcaacacaaaacaacgatcaaagttcttccttttttatggaaccaaagttgtttctttggagtgccatagttggaatcgtgtttggtgtttctaatttcatgtacgcattgggtttatcttatcttccagtatcaacttcgacaattctctttgcaactcaactgtgtttcacagcaatttttgcatggttaattgtgaaacaaaaatttacagcatttattataaatgcagtgattgtaatgacactaggatcgatcttattgggtattaataccaatggtgatagaccaattggggtatcaaaaactcagtacttaatagggtttcttatgacgttagctgctgctgctctaactggcctcgggacgccttttgttgagctttctttcattaaagccaccagaaatattacttatccaactttgttacagtttcaagtcattctttgtctgtttggaacctgcctcaacgtcattgggatgctaataaataaggattttcaggctatacccagagaagcagacatgttcgagcttgggaaaagcaagtattatatgataatatgcttgactgcattgacatggcaattatcaggaattggactcgtaggcctaattttgtacacaaatgctcttttcaacggtatatacgtatccgttcttgttccgttcacagaagttgcagcggtcatatttttccatgagaagtttacgggattaaagggaatggcattggcattatgtctttggggtttctcttcctatttctatggagaatacaagatgatgaataaagtgggtgataatgaaacacatgagaaaatcgaggaagccgaaagcgagcccaaaagattagaggatcaacaagcaccatacagtactgtatga

SEQ ID NO: 37 - protein, 284 aa, Papaver somniferum
MIIETLDILGPNQNGNSGTHTQKPIKTRNWLLIIINCALVFCGVIGGPLLMRLYYLHGGSRKWLSSFLQTAGFPVLIFPLIFLYIKPKLSTQNNDQSSSFFMEPKLFLWSAIVGIVFGVSNFMYALGLSYLPVSTSTILFATQLCFTAIFAWLIVKQKFTAFIINAVIVMTLGSILLGINTNGDRPIGVSKTQYLIGFLMTLAAAALTGLGTPFVELSFIKATRNITYPTLLQFQVILCLFGTCLNVIGMLINKDFQVRNCYRRLTTFLIFLILEQKLISEEDL

SEQ ID NO: 38 - DNA, 825 bp, Papaver somniferum
atgatcatcgaaacactagatatcctgggaccaaatcagaatggcaattcaggaacccatactcaaaaaccaatcaaaaccagaaactggctgctgatcattattaactgcgccttagttttttgtggtgttataggtggtcctctcttaatgagactgtactatcttcatggtggtagtcgtaaatggcttagtagttttctgcaaactgctggtttcccagttctcatatttcctctcatttttctctacattaaaccgaaattgtcaacacaaaacaacgatcaaagttcttccttttttatggaaccaaagttgtttctttggagtgccatagttggaatcgtgtttggtgtttctaatttcatgtacgcattgggtttatcttatcttccagtatcaacttcgacaattctctttgcaactcaactgtgtttcacagcaatttttgcatggttaattgtgaaacaaaaatttacagcatttattataaatgcagtgattgtaatgacactaggatcgatcttattgggtattaataccaatggtgatagaccaattggggtatcaaaaactcagtacttaatagggtttcttatgacgttagctgctgctgctctaactggcctcgggacgccttttgttgagctttctttcattaaagccaccagaaatattacttatccaactttgttacagtttcaagtcattctttgtctgtttggaacctgcctcaacgtcattgggatgctaataaataaggattttcaggtacgtaactgttataggaggcttacaacctttttgattttccttattctctga

SEQ ID NO: 39 - DNA, 855 bp, Papaver somniferum
atgatcatcgaaactttggatatcttgggtccaaaccaaaacggtaactcaggtactcatacacaaaaaccaattaaaacaagaaactggttgttgatcattattaactgtgctttagttttctgtggtgttattggtggtccattgttgatgagattgtactacttgcatggtggttctagaaagtggttatcttcatttttgcaaactgcaggttttccagttttgatcttcccattgattttcttgtacattaaaccaaaattgtcaacacaaaacaacgatcaatcttcttctttctttatggaaccaaagttgtttttatggtctgctattgttggtatcgttttcggtgtttcaaacttcatgtacgcattgggtttgtcttacttgccagtttcaacttctacaatcttgttcgctactcaattgtgtttcacagctatcttcgcatggttgatcgttaagcaaaagtttactgcttttattattaatgcagttattgttatgactttgggttcaatcttgttgggtattaatacaaacggtgacagaccaatcggtgtttctaagactcaatatttgatcggtttcttgatgacattggctgcagctgcattaactggtttgggtacaccatttgttgaattgtcttttattaaggctactagaaacatcacttacccaacattgttgcaattccaagttattttgtgtttgttcggtacatgtttgaacgttatcggcatgttgattaataaggatttccaagttagaaactgttacagaagattgacaacattcttgatcttcttgatcttggaacaaaaattaatttctgaagaagatttgtaa

SEQ ID NO: 40 - protein, 10 aa, Artificial Sequence
  Myc-Tag
EQKLISEEDL

SEQ ID NO: 41 - protein, 356 aa, Arabidopsis thaliana
MKNGLIIINCIILTIGTCGGPLLTRLYFTNGGKRIWFMSFLSTAGFPIILIPLLVSFLSRRRSNRNPNNAENKRKTKLFLMETPLFIASIVIGLLTGLDNYLYSYGLAYLPVSTSSLIIGTQLAFNALFAFLLVKQKFTPFSINAVVLLTVGIGILALHSDGDKPAKESKKEYVVGFLMTVVAALLYAFILPLVELTYKKARQEITFPLVLEIQMVMCLAATFFCVIGMFIVGDFKVIAREAREFKIGGSVFYYALIVITGIIWQGFFLGAIGIVFCASSLASGVLISVLLPVTEVFAVVCFREKFQAEKGVSLLLSLWGFVSYFYGEFKSGKKVVDKPQPPETELPILPVSDYVA

SEQ ID NO: 42 - DNA, 1071 bp, Arabidopsis thaliana
atgaagaacggtttgattattattaactgcattattttgactatcggtacatgtggtggtcctttattgacaagattatactttaccaatggtggtaaaagaatttggttcatgtcatttttgtcaactgctggtttcccaatcatcttgatcccattgttggtttcatttttgtcaagaagaagatctaacagaaacccaaacaatgcagaaaacaagagaaagactaaattatttttgatggaaacaccattattcatcgcttcaatcgttatcggtttgttgacaggtttagataactacttgtactcttatggtttagcatacttgccagtttcaacttcttcattgatcatcggtacacaattagctttcaacgcattgttcgcatttttgttggttaagcaaaagttcactccattctctatcaacgctgttgttttgttgacagttggtatcggtattttagcattgcattctgatggtgataagccagctaaggaatctaaaaaagaatatgttgttggtttcttgatgactgttgttgctgcattgttgtacgcattcatcttgccattggttgaattgacttacaagaaggctagacaagaaatcacattcccattagttttggaaatccaaatggttatgtgtttagctgcaactttcttttgtgttatcggcatgttcatcgttggtgatttcaaggttatcgcaagagaagctagagaatttaagatcggtggttctgttttctattacgcattgatcgttattactggtattatttggcaaggtttctttttgggtgctattggtattgttttctgtgcatcttcattagcttctggtgttttgatttcagttttgttaccagttacagaagttttcgcagttgtttgtttcagagaaaagttccaagctgaaaagggtgtttctttgttgttgtcattgtggggttttgtttcttacttttatggtgaatttaaatcaggtaaaaaagttgttgacaaacctcaaccaccagaaaccgaattacctatcttaccagtctccgattatgtagcataa

SEQ ID NO: 43 - protein, 345 aa, Jatropha curcas
MRRALLVLNCVILSIGNCGGPLIMRLYFIHGGKRVWLSSWLETAGWPIIFIPLLISYFHRRSTTDPTTAKLFYMKPSLFLAATGIGILTGFDDYLYAYGVARLPVSTSSLIIATQLAFTAGFAFLLVKQKFTSYSINAVVLLTVGAGVLALHTSSDRPEHESKKEYNLGFVMTLGAAVLYGLILPLVELTYRKAKQEISYTLVMEIQMIMCLFATVVCTVGMLVNNDFKVIPREAKEFELGETKYYVIMVWSAIIWQCFFLGAIGIVFCASSLASGVVIAVLLPVTEILAVIFYQEKFQAEKGVALALSLWGFLSYFYGEIKQSKKTNLTSEIETSESSIPTQNV

SEQ ID NO: 44 - DNA, 1038 bp, Jatropha curcas
atgagaagagctttgttagttttgaactgtgttatcttgtctatcggtaattgtggtggtccattgatcatgagattgtacttcattcatggtggtaaaagagtttggttgtcttcatggttagaaactgctggttggccaatcatcttcatcccattgttaatttcttactttcatagaagatcaactacagatccaactacagcaaaattgttttatatgaagccatctttgtttttagctgcaactggtattggtattttgacaggtttcgatgattacttgtacgcttatggtgttgctagattgccagtttcaacttcttcattgatcatcgctactcaattagcttttacagcaggttttgcatttttgttggttaagcaaaagttcacatcttactcaatcaatgcagttgttttgttaactgttggtgcaggtgttttggctttacatacatcttcagatagaccagaacatgaatctaaaaaagaatacaacttgggttttgttatgacattgggtgctgctgttttgtacggtttgatcttgccattggttgaattaacttacagaaaggctaagcaagaaatttcatacacattggttatggaaattcaaatgatcatgtgtttgttcgcaactgttgtttgtacagttggcatgttggttaacaacgatttcaaggttatcccaagagaagctaaggaatttgaattaggtgaaactaagtattacgttattatggtttggtctgcaattatttggcaatgtttctttttgggtgctattggtattgttttctgtgcatcttcattagcttcaggtgttgttattgcagttttgttaccagttacagaaattttggctgttattttctatcaagaaaagttccaagcagaaaagggtgttgctttagcattgtctttatggggtttcttgtcatacttttatggtgaaatcaagcaatctaagaaaactaacttgacatctgaaatcgaaacttcagaatcttcaatcccaacacaaaatgtttaa

SEQ ID NO: 45 - protein, 350 aa, Papaver somniferum
MGKYLIFCCMLLLVGQVGGPLLLRLYYLHGGQRKWLTSWLQTAAFPILLIPILVSWSKSKSKSQSISTNAVNPTDHRNLFCVTRKLFISSVILGIMFGLDAFLFSIGLSNLPVSTSTLLMATQLAFTVFFASILVKQKFTPYSINSVVLLTLGAVVLAFHTNGDKPIGVSKDQYFLGFFVTLGAAALFGFMLPFIELVYRKACEAVTYDLVMRMQFITSMVATVFCTIAMLINKDFQAISREAKGFELGETKYYIVLIFTAVSMQCAVVGTLGVIHCASSLFSGVLMTLLLPIQQICAIFFFNEKFSAEKGMSLGLSIWGFASYFYGEYKQTKKKTHQHKAVSTKSQEIP

SEQ ID NO: 46 - DNA, 1053 bp, Papaver somniferum
atgggcaagtacttgattttctgttgtatgttgttattggttggtcaagttggtggtccattgttgttgagattgtactacttgcatggtggtcaaagaaaatggttaacttcttggttgcaaacagctgcattcccaatcttgttgatcccaattttagtttcttggtcaaaatctaaatcaaagtctcaatcaatttctactaacgctgttaacccaacagatcatagaaacttattttgtgttactagaaaattgtttatttcttcagttattttaggtatcatgttcggtttagatgcatttttgttttcaatcggtttatctaacttgccagtttcaacttctacattgttaatggcaactcaattggcttttacagttttctttgcttcaattttagttaagcaaaagttcactccatattcaattaattctgttgttttgttaactttaggtgcagttgttttggcttttcatacaaatggtgataagccaatcggtgtttctaaggatcaatactttttgggtttctttgttacattaggtgctgctgctttgtttggtttcatgttgccattcatcgaattggtttatagaaaagcatgtgaagctgttacttacgatttggttatgagaatgcaattcatcacatcaatggttgcaactgttttctgtacaatcgctatgttgatcaacaaggattttcaagctatttcaagagaagctaagggtttcgaattgggtgaaactaagtactacatcgttttgatcttcacagcagtttcaatgcaatgtgctgttgttggtactttaggtgttatccattgtgcttcttcattattttctggtgttttgatgacattgttgttgccaatccaacaaatttgtgcaattttctttttcaatgaaaagttctcagctgaaaagggcatgtcattgggtttgtctatttggggtttcgcatcttacttctacggtgaatacaagcaaactaaaaagaaaactcatcaacataaggctgtttcaacaaagtctcaagaaattccataa

SEQ ID NO: 47 - protein, 348 aa, Papaver somniferum
MGKYLLLFNCILLAVSSAGGPLLLRLYFIHGGKRLWLSSWLETAGWPILFLPLSLSYFLKRRRFKNGQDEKPSKFFMITPFLFMASAFIGLLVGLDDYLYTYGVSLLPVSTSALIMSTHLAFTAGFALFMVKQKFTSYSVNAVILLTVGAILLGLHSNGDTPVHESNRDYYLGFVMTIGASIIGGLLLPLVELMYKKSKQTITYSLVIELQIVISVFATLLCTVGMLVNNDFKVIQREGKEYELGETNYYVVLVASSITWQLCYLGTIGVIFCSTSLLAGVIGAVVLPVIEILAVIFYHESFKAEKGIALFLSLWGFISYFYLEIKESTKPKKKRSLELEQGDLTVSS

SEQ ID NO: 48 - DNA, 1047 bp, Papaver somniferum
atgggcaagtacttgttgttgttcaactgtatcttattggcagtttcttcagctggtggtccattgttgttgagattgtacttcattcatggtggtaaaagattatggttgtcttcatggttagaaacagcaggttggccaatcttatttttgccattatctttgtcatactttttgaagagaagaagattcaagaatggtcaagatgaaaaaccatctaagtttttcatgatcactccatttttattcatggcttcagcattcattggtttgttagttggtttggatgattacttgtacacttatggtgtttctttgttaccagtttctacttcagcattgatcatgtcaactcatttggctttcacagcaggttttgctttgttcatggttaagcaaaagttcacatcttactcagttaatgcagttatcttgttgactgttggtgctatcttgttaggtttgcattctaatggtgatacaccagttcatgaatcaaacagagattactacttgggtttcgttatgactatcggtgcttctatcattggtggtttgttgttgccattggttgaattaatgtacaaaaaatctaagcaaactattacatattcattggttattgaattacaaattgttatttctgtttttgcaactttgttgtgtacagttggcatgttggttaacaacgatttcaaggttatccaaagagaaggcaaggaatacgaattgggtgaaacaaactactacgttgttttagttgcttcttcaatcacttggcaattgtgttacttgggtacaatcggtgttattttctgttctacttcattattggcaggtgttattggtgctgttgttttgccagttatcgaaattttagctgttattttctatcatgaatcttttaaggcagaaaagggtatcgctttatttttgtctttatggggtttcatctcatacttctatttggaaatcaaagaatctacaaagccaaaaaagaaaagatcattggaattggaacagggtgatttaactgtttcttcataa

SEQ ID NO: 49 - protein, 329 aa, Papaver somniferum
MGKYLLLRLYYLHGGQRKWLSSWLQTVAFPFLLIPISVSWFKSKSKSHDSRSISAIDVNPTTDRKLRFGGFSPKLFISCIFLGIIVGLDSFLYAYGVSYLPVSTSSLLMSTQLAFTAAFALLLVRQKFTPYSINSVVLLTLGAVVLAFHTNGDKPIGVSKDQYFLGFFVTLGAAALFGFMLPFIELVYRKACEAVTYDLVMRMQFIISMVATVFCTIAMLINKDFQAISREAKGFELGETKYYIVLIFTAVSMQCAVVGTLGVIHCASSLFSGVLMTLLLPIQQICAIFFFNEKFSAEKGMSLGLSIWGFASYFYGEYKQTEKKTNQHK

SEQ ID NO: 50 - DNA, 990 bp, Papaver somniferum
atgggcaagtacttgttgttgagattgtactacttgcatggtggtcaaagaaaatggttatcttcatggttgcaaactgttgcattcccatttttattgatcccaatttctgtttcatggttcaagtctaagtcaaagtctcatgattcaagatcaatttctgctatcgatgttaacccaactacagatagaaaattgagattcggtggtttctctccaaaattgttcatctcatgtattttcttgggtatcatcgttggtttagattcatttttgtacgcttacggtgtttcttacttgccagtttcaacttcttcattattgatgtcaactcaattggcatttacagctgcattcgctttgttgttagttagacaaaagttcacaccatactctatcaactcagttgttttgttgactttgggtgcagttgttttggcttttcatacaaatggtgataagccaatcggtgtttctaaggatcaatactttttgggtttctttgttactttaggtgctgctgctttgtttggtttcatgttgccattcatcgaattggtttatagaaaagcatgtgaagctgttacatacgatttggttatgagaatgcaattcatcatctctatggttgcaactgttttctgtacaatcgctatgttgatcaacaaggattttcaagctatttcaagagaagctaagggtttcgaattaggtgaaactaagtactacatcgttttgatcttcacagcagtttctatgcaatgtgctgttgttggtactttgggtgttatccattgtgcatcttcattattttcaggtgttttgatgacattgttgttgccaatccaacaaatttgtgcaattttctttttcaatgaaaagttctctgctgaaaagggcatgtctttgggtttgtcaatttggggtttcgcttcatacttctacggtgaatacaaacaaactgaaaagaaaactaatcaacataaataa

SEQ ID NO: 51 - protein, 384 aa, Papaver somniferum; identical to SEQ ID NO: 35

SEQ ID NO: 52 - DNA, 1155 bp, Papaver somniferum
atgatcatcgaaactttggatatcttgggtccaaaccaaaacggtaactcaggtactcatacacaaaaaccaattaaaacaagaaactggttgttgatcattattaactgtgctttggttttctgtggtgttattggtggtccattgttgatgagattgtactacttgcatggtggttctagaaagtggttgtcttcatttttgcaaactgcaggttttccagttttgatcttcccattgattttcttgtacattaaaccaaaattgtcaacacaaaacaacgatcaatcttcatctttctttatggaaccaaagttgtttttatggtctgctattgttggtatcgttttcggtgtttcaaacttcatgtacgcattgggtttatcttacttgccagtttcaacttctacaatcttgttcgctactcaattgtgtttcacagctatcttcgcatggttgatcgttaagcaaaagtttactgcttttattattaatgcagttattgttatgactttgggttcaatcttgttgggtattaatacaaacggtgacagaccaatcggtgtttctaagactcaatatttgatcggtttcttgatgacattggctgcagctgcattaactggtttgggtacaccatttgttgaattgtcttttattaaggctactagaaacatcacttacccaacattgttgcaattccaagttattttgtgtttgttcggtacatgtttgaacgttatcggcatgttgattaataaggatttccaagctatcccaagagaagcagatatgtttgaattgggtaaatcaaagtactacatgatcatctgtttaactgctttgacatggcaattatctggtattggtttggttggtttgatcttgtacacaaacgcattgtttaatggtatctatgtttctgttttggttccttttactgaagttgctgctgttattttctttcatgaaaagtttactggtttaaagggtatggctttggcattgtgtttgtggggtttttcatcttacttctacggtgaatacaagatgatgaataaggttggtgacaatgaaactcatgaaaagattgaagaagctgaatcagaaccaaaaagattggaagatcaacaagcaccatactctacagtttaa

SEQ ID NO: 53 - protein, 348 aa, Papaver alpinum
MNTYLLLFNGILLAVSSIAGPLLLRLYFIHGGKRIWLSSCLETAGFPVLIFPLWLSYFLRRRGFIKGDDDEKPKKLFTITLPLFIASAVIGLVTGLDDYLYTYGVSLLPISTATIIMSTHLAFTAGFALVMVKQKFTSFSVNAVVLLTIGAILLGLHGNGDKPVNESKKDYYLGFLITIAASVFNGLMLPMVELMYMKSKQTITYSLVIELQMVISGFATLFCTIGMIANNDFKVIPREGREYGLGEINYYIVLVASAITWQMYFVGTVGVIFCSTSLHAGVISVVVLPLTEILSVVFYHESFKAEKGIALFLSLWGFISYFYLEIKASRKPKKQCSELEQGGLTVSS

SEQ ID NO: 54 - DNA, 1047 bp, Papaver alpinum
atgaatacatacttgttgttgttcaacggtattttattggcagtttcttcaattgctggtccattgttgttgagattgtacttcattcatggtggtaaaagaatttggttatcttcatgtttggaaactgctggttttccagttttgatcttcccattgtggttgtcttactttttaagaagaagaggtttcatcaagggtgatgatgatgaaaagcctaaaaaattgttcactatcacattgccattgttcatcgcttcagcagttatcggtttagttactggtttggatgattacttgtacacttatggtgtttctttgttgccaatttcaactgctacaatcatcatgtctactcatttggcttttacagcaggttttgctttagttatggttaagcaaaagttcacatctttttcagttaacgcagttgttttgttgactatcggtgctatcttgttaggtttgcatggtaatggtgataaaccagttaacgaatctaaaaaagattactacttaggtttcttgatcacaatcgctgcatcagttttcaacggtttgatgttgccaatggttgaattgatgtacatgaagtctaagcaaactatcacatactcattggttatcgaattacaaatggttatttctggtttcgcaactttattttgtacaattggtatgatcgctaacaacgatttcaaggttattccaagagaaggtagagaatacggtttgggtgaaatcaactactacatcgttttagttgcttctgcaattacttggcaaatgtattttgttggtacagttggtgttattttctgttctacttcattgcatgcaggtgttatttcagttgttgttttgccattgacagaaattttatctgttgttttctatcatgaatcatttaaggcagaaaagggtatcgctttgtttttatctttgtggggtttcatctcatacttctatttagaaatcaaagctagtagaaagcctaaaaaacaatgttcagaattggaacaaggtggtttaactgtttcttcataa

SEQ ID NO: 55 - protein, 347 aa, Papaver atlanticum
MEKYLLLFNCILLAVCSAGGPLLLRLYFIHGGKRLWLSSWLETAGWPILFLPLSLSYFLKRRRFKNGQDEKPSKFFMITPFLFMASAFIGLLVGLDDYLYTYGVSLLPVSTASLIMSTHVAFTAGFALFMVKQKFTSYSVNAVILLTVGAVLLGLHSNGDRSVHESNRDYYLGFVMTIGASVIGGLLLPLVELMYKKSKQTITYTLVTELQIVISVFATLFCTVGMLVNNDFKVIQREGKEYDLGETKYYVVLVASSITWQLCFLGTIGVIFCSTSLLAGVIGAAVLPVIEILGVIFYHESFKAEKGIALFLSLWGFISYFYLEIKASRKPKRQCSELEQGGLTVSS

SEQ ID NO: 56 - DNA, 1044 bp, Papaver atlanticum
atggaaaagtacttgttgttgttcaactgtatcttattggcagtttgttcagctggtggtccattgttgttgagattgtacttcattcatggtggtaaaagattatggttgtcttcatggttggaaactgctggttggccaatcttatttttgccattatctttgtcatactttttgaagagaagaagattcaagaatggtcaagatgaaaaaccatctaagtttttcatgatcacaccatttttattcatggcttcagcattcattggtttgttagttggtttggatgattacttgtacacttatggtgtttctttgttaccagtttctacagcttcattgattatgtcaacacatgttgcttttactgctggtttcgctttgttcatggttaagcaaaagtttacttcttattcagttaatgcagttattttgttaacagttggtgctgttttgttaggtttgcattctaatggtgatagatcagttcatgaatcaaacagagattactacttgggtttcgttatgactattggtgcatctgttattggtggtttgttgttgccattggttgaattaatgtacaaaaaatcaaagcaaactattacatatactttggttacagaattacaaattgttatttctgtttttgctacattgttttgtactgttggcatgttggttaacaacgatttcaaggttatccaaagagaaggcaaggaatacgatttgggtgaaactaaatactacgttgttttagttgcatcttcaattacatggcaattgtgtttcttgggtactatcggtgttattttctgttctacatcattattggctggtgttattggtgctgctgttttgccagttatcgaaattttaggtgttattttctatcatgaatcttttaaggcagaaaagggtatcgctttatttttgtctttatggggtttcatctcatacttctatttggaaatcaaagctagtagaaagccaaagagacaatgttcagaattggaacaaggtggtttaacagtttcttcataa

SEQ ID NO: 57 - protein, 351 aa, Papaver miyabeanum
MEKYLLLFNCILLAVGSTAGPLLLRLYFIHGGKRLWLSSWLETAGWPILFLPLSLSYFLKRRRFKTGQDEKPSKFFMITPFLFMASAFIGILVGLDDYLYTYGVSLLPVSTSALIMSTHLAFTAGFALFMVKQKFTSYSVNAVVLLTVGAILLGLHSNGDRPLYESNRDYYLGFVMTIGASVIGGLLTPLVELMYKKSKQTITYTLVIELQIVMSVFATLFCTVGMLVNNDFKVIQREGKEYDLGETKYYVVLVASSITWQLCFLGIVGVVFCSTSLLAGVIGAVVVPVIEILGVIFYHESFKAEKGIALFLSLWGFISYFYLELKEIKKPKNHHSELEEDLTVSSQSNLA

SEQ ID NO: 58 - DNA, 1056 bp, Papaver miyabeanum
atggaaaagtacttgttgttgttcaactgtatcttattggcagttggttctacagctggtccattgttgttgagattgtacttcattcatggtggtaaaagattgtggttatcttcatggttggaaactgctggttggccaatcttgtttttaccattgtctttatcatactttttgaagagaagaagattcaagacaggtcaagatgaaaagccatctaagtttttcatgatcactccatttttattcatggcttcagcattcatcggtattttagttggtttggatgattacttgtacacttatggtgtttctttgttaccagtttctacttcagcattgatcatgtcaacacatttggctttcactgctggtttcgctttgttcatggttaagcaaaagtttacatcttactcagttaatgcagttgttttgttaactgttggtgctatcttgttgggtttacattctaacggtgatagaccattgtacgaatcaaacagagattactacttgggtttcgttatgacaattggtgcttctgttattggtggtttgttgactccattagttgaattgatgtacaaaaaatcaaagcaaactatcacatacactttagttattgaattgcaaatcgttatgtctgttttcgcaacattattttgtactgttggcatgttggttaacaacgatttcaaggttatccaaagagaaggcaaggaatacgatttgggtgaaacaaagtactacgttgttttggttgcttcttcaatcacttggcaattgtgtttcttgggtattgttggtgttgttttctgttctacatcattgttagcaggtgttattggtgctgttgttgttccagttatcgaaattttaggtgttattttctatcatgaatcttttaaggcagaaaagggtatcgctttgtttttatctttgtggggtttcatctcatacttctatttagaattgaaagaaattaagaaaccaaaaaatcatcattctgaattagaagaagatttgactgtttcttcacaatcaaacttggcttaa

SEQ ID NO: 59 - protein, 355 aa, Papaver nudicale
MNTCLLWFNGLLLAISSIGGPLLLRLYFIHGGKRIWLSSCLETAGFPVLFLPLWLSYFLKRRGVIKGDEGEKPSKLFTITRPLFIASAGIGLITGLDDYLYTYGVSLLPISTATIIMSTHLAFTAGFALVMVKQKFTSFSVNAVVLLTVGAILLGLHSNGDRPANESTKEYYLGFLITIAASVINGLMLPLVELMYMKSKQVITYSLVIELQIVISAFATLFCTIGMIVDNDFKVIPREGREYGLGEVNYYVVLVSSAIMWQMYFVGTVGVIFCSTSLLAGVIAVVVLPLTEILSVVFYHESFKAEKGIALFLSLWGFISYFWGELKGSRKAKKQISELEQDSSNSPTSLHILDY

SEQ ID NO: 60 - DNA, 1068 bp, Papaver nudicale
atgaatacttgtttgttgtggttcaacggtttgttattggcaatttcttcaatcggtggtccattgttgttgagattgtacttcattcatggtggtaaaagaatttggttgtcttcatgtttagaaacagctggttttccagttttgtttttaccattgtggttgtcttactttttgaagagaagaggtgttatcaagggtgatgaaggtgaaaagccatctaaattgttcactatcacaagaccattgttcatcgcttcagcaggtatcggtttgatcactggtttagatgattacttgtacacttatggtgtttctttgttgccaatttcaactgcaacaatcatcatgtctactcatttggcttttacagcaggttttgctttggttatggttaagcaaaagttcacttctttttcagttaacgcagttgttttgttaacagttggtgctatcttgttgggtttacattctaacggtgatagaccagctaacgaatcaactaaggaatactacttgggtttcttgatcacaatcgctgcatctgttatcaacggtttgatgttgccattggttgaattaatgtacatgaagtctaagcaagttatcacttactcattagttattgaattgcaaatcgttatttcagctttcgcaactttgttttgtacaatcggtatgatcgttgataacgatttcaaggttattccaagagaaggtagagaatacggtttaggtgaagttaactactacgttgttttggtttcttcagcaattatgtggcaaatgtattttgttggtactgtcggtgttattttctgttctacatcattgttagcaggtgttattgctgttgttgttttgccattgactgaaattttgtctgttgttttctatcatgaatcatttaaggcagaaaagggtatcgctttatttttgtctttatggggtttcatctcatacttctggggtgaattaaaaggttcaagaaaggctaaaaaacaaatttcagaattggaacaagattcttcaaattctccaacatcattgcatattttagattactaa

SEQ ID NO: 61 - protein, 341 aa, Papaver radicatum
MKKSLMLFNTILLGIGATGGPLLLRLYFVRGGKRIWLSSALGSAGWPVLILPLSLSYFFNRGGRGGDKRWYKFYTITPPLIVFSAFIGIILGSNDYLYTHGISLLPVSTSTLIMSTHLAFTAGFAFVIVKHKFTPYSINAVVLLTVGAVLLGLNSSGDKPVNQSKKDYYLGFFLTVGASVISGFLFPLSELMYMKAKERLTYSLVIEMQIVTAVVASLFCIVGMIVNNDFQAIPREGRDYELGEVKYYVVLVAIAIMWQIYFVGTAGVIFCSTSLYAGIITAVILPVTEILSVVFYHESFKSEKGLALFLSCWGFISYLYGDYKENLKLKKAQKQSSEMEL

SEQ ID NO: 62 - DNA, 1026 bp, Papaver radicatum
atgaaaaaatcattaatgttgttcaacactatcttgttgggtatcggtgcaacaggtggtccattgttgttgagattgtacttcgttagaggtggtaaaagaatttggttatcttcagcattgggttctgctggttggccagttttgatcttgccattatctttgtcatatttctttaatagaggtggtagaggtggtgataagagatggtacaagttctacactatcacaccaccattgatcgttttctctgctttcatcggtatcatcttgggttcaaacgattacttgtacactcatggtatttctttattgccagtttctacttcaacattgatcatgtcaactcatttggcttttacagcaggtttcgctttcgttatcgttaagcataagtttactccatattcaattaatgcagttgttttattgacagttggtgctgttttgttgggtttaaattcttcaggtgataagccagttaaccaatctaaaaaagattactacttaggtttctttttgacagttggtgcatctgttatttcaggtttcttgttcccattgtctgaattgatgtacatgaaggctaaggaaagattgacttactcattggttatcgaaatgcaaatcgttacagcagttgttgcttctttattttgtatcgttggtatgatcgttaataatgattttcaagcaattccaagagaaggtagagattacgaattaggtgaggttaagtactacgttgttttggttgctatcgcaatcatgtggcaaatttatttcgttggtactgctggtgttattttctgttctacatcattgtacgcaggtatcatcactgctgttatcttgccagttacagaaattttgtctgttgttttctatcatgaatcttttaagtcagaaaaaggtttagcattgtttttatcttgttggggtttcatctcatacttatacggtgattacaaggaaaacttgaaattgaaaaaagctcaaaaacaatcttcagaaatggaattgtaa

SEQ ID NO: 63 - protein, 348 aa, Papaver trinifolium
MGKYLLLFNCILLAVSSAAGPLLLRLYFIHGGKRLWLLSWLETAGWPILFLPLSLSYFLKRRRFKNGQDEKPSKFFMITPFLFMASAFIGLLIGLDDYLYTYGVSLLPVSTSALIMSTHLAFTAGFALFMVKQKFTSYSVNAVILLTVGAVLLGLHSNGDKPVHESNRDYYLGFVITIGASVIGGLLLPLVELMYKKSKQTITYSLVIELQIVISVFATLFCTVGMLVNNDFKVIQREGKEYNLGETKYYVVLVASSISWQLCFLGTIGVIFCSTSLLAGVIGAVVLPVIEILAVIFYHESFKAEKGIALFLSLWGFISYFYLELKASRKPKKKQSLELEQGDLTVSS

SEQ ID NO: 64 - DNA, 1047 bp, Papaver trinifolium
atgggcaagtacttgttgttgttcaactgtatcttgttggctgtttcttctgctgctggtccattgttgttgagattgtacttcattcatggtggtaaaagattgtggttgttatcttggttagaaactgctggttggccaatcttatttttgccattatctttgtcatactttttgaagagaagaagattcaagaatggtcaagatgaaaaaccatctaagtttttcatgatcacaccatttttattcatggcttcagcattcatcggtttgttgatcggtttggatgattacttgtacacttatggtgtttctttgttaccagtttctacatcagcattgatcatgtcaactcatttggctttcacagcaggtttcgctttgttcatggttaagcaaaagtttacttcttattcagttaatgcagttattttgttaacagttggtgctgttttgttaggtttgcattctaatggtgataagccagttcatgaatcaaacagagattactacttgggtttcgttatcactatcggtgcttctgttattggtggtttgttgttgccattggttgaattaatgtacaaaaaatctaagcaaactattacatattcattggttattgaattacaaattgttatttcagtttttgcaactttgttttgtacagttggcatgttggttaacaacgatttcaaggttattcaaagagaaggcaaggaatacaacttgggtgaaacaaagtactacgttgttttagttgcttcttcaatttcttggcaattgtgtttcttgggtactatcggtgttattttctgttctacatcattattggcaggtgttattggtgctgttgttttgccagttatcgaaattttagcagttattttctatcatgaatcttttaaggcagaaaagggtatcgctttatttttgtctttatggggtttcatctcatacttctatttggaattaaaagctagtagaaagccaaagaaaaaacaatcattggaattagaacagggtgatttgactgtttcttcataa

SEQ ID NO: 65 - DNA, 20 bp, Artificial Sequence
  qRT-PCR forward primer for THS2F
gaatccccggccaacctatc

SEQ ID NO: 66 - DNA, 21 bp, Artificial Sequence
  qRT-PCR reverse primer for THS2
acctgaaacaccgagaggagc

SEQ ID NO: 67 - DNA, 28 bp, Artificial Sequence
  qRT-PCR forward primer for THS2S
taacagctaatcctgaacagtttagtcg

SEQ ID NO: 68 - DNA, 21 bp, Artificial Sequence
  qRT-PCR reverse primer for THS2S2
cgcaaagatgaggaactgcct

SEQ ID NO: 69 - DNA, 24 bp, Artificial Sequence
  qRT-PCR forward primer for THS1
gcaacatgccaaagttagaacagc

SEQ ID NO: 70 - DNA, 21 bp, Artificial Sequence
  qRT-PCR reverse primer for THS1
gaaacaccgagaggagccatc

SEQ ID NO: 71 - DNA, 22 bp, Artificial Sequence
  qRT-PCR forward primer for THS1S
gcaacatgccaaagtctagtcg

SEQ ID NO: 72 - DNA, 20 bp, Artificial Sequence
  qRT-PCR reverse primer for THS1S
aacctgaacgggttgggtct

SEQ ID NO: 73 - DNA, 29 bp, Artificial Sequence
  genomic PCR forward primer for BV1 (5' UTR)
tgggctcatatgtgacactgcttaaccac

SEQ ID NO: 74 - DNA, 32 bp, Artificial Sequence
  genomic PCR forward primer for BV1 (5' UTR) (THS1)
ttacatcaattctttatagcaacatgccaaag

SEQ ID NO: 75 - DNA, 30 bp, Artificial Sequence
  genomic PCR forward primer for BV1 (5' UTR) (nested)
acaacgggactatactactaataccgaatc

SEQ ID NO: 76 - DNA, 28 bp, Artificial Sequence
  genomic PCR reverse primer for BV1 (5' UTR)
tatgtacgtgcataggtacacgtacacc

SEQ ID NO: 77 - DNA, 20 bp, Artificial Sequence
  VIGS forward primer - TRV2
ggtcaaggtacgtagtagag

SEQ ID NO: 78 - DNA, 21 bp, Artificial Sequence
  VIGS reverse primer - TRV2
cgagaatgtcaatctcgtagg

SEQ ID NO: 79 - DNA, 249 bp, Artificial Sequence
  Synthetic VIGs fragment - TRV2
aatgttaacattgatggtaagacgattcgctcggtacaattcggccatcaggccattgaggacatgaacaagtacttacgcgattctgaaagtaactgattgatgccatttatacatgaacccattcggtgttggtgtacgtgtacctatgcacgtacatattttatatttatcagttgcaacttgtgtgtattttatcgtttcagtgactccaatattgtgtcagtgacccggtgtatgggtgtgatt

SEQ ID NO: 80 - protein, 180 aa, Papaver somniferum
MDSINSSIYFCAYFRELIIKLLMAPLGVSGLVGKLSTELEVDCDAEKYYNMYKHGEDVQKAVPHLCVDVKVISGDPTRSGCIKEWNVNIDGKTIRSVEETTHNDETKTLRHRVFEGDMMKDFKKFDTIMVVNPKPDGNGCVVTRSIEYEKTNENSPTPFDYLQFGHQAIEDMNKYLRDSE

SEQ ID NO: 81 - protein, 130 aa, Papaver somniferum
MYKHGEDVQKAVPHLCVDVKVISGDPTRSGCIKEWNVNIDGKTIRSVEETTHNDETKTLRHRVFEGDMMKDFKKFDTIMVVNPKPDGNGCVVTRSIEYEKTNENSPTPFDYLQFGHQAIEDMNKYLRDSE